European Patent Application EP 4 494 639 A1, published January 22, 2025. Title: Alox5 억제제를 포함하는 근감소증 예방 또는 치료용 조성물. Applicant: 광주과학기술원. Application KR. The sequence listing filed with the application follows.

SEQUENCE LISTING (26 sequences)

SEQ ID NO: 1 - DNA, 20 bp, Artificial Sequence
  source 1..20: mol_type = unassigned DNA
ctccactcacggcaaattca

SEQ ID NO: 2 - DNA, 20 bp, Artificial Sequence
  source 1..20: mol_type = unassigned DNA
gcctcaccccatttgatgtt

SEQ ID NO: 3 - DNA, 20 bp, Artificial Sequence
  source 1..20: mol_type = unassigned DNA
cagagagctgctccgtctca

SEQ ID NO: 4 - DNA, 19 bp, Artificial Sequence
  source 1..19: mol_type = unassigned DNA
acgtatcccccgcagtttc

SEQ ID NO: 5 - DNA, 21 bp, Artificial Sequence
  source 1..21: mol_type = unassigned DNA
ccgagtgcagacgatcatctc

SEQ ID NO: 6 - DNA, 20 bp, Artificial Sequence
  source 1..20: mol_type = unassigned DNA
tggaggatcagagcctcgat

SEQ ID NO: 7 - DNA, 22 bp, Artificial Sequence
  source 1..22: mol_type = unassigned DNA
tggagtccatcatccgtagtga

SEQ ID NO: 8 - DNA, 23 bp, Artificial Sequence
  source 1..23: mol_type = unassigned DNA
ctggtacccagctttgagatgag

SEQ ID NO: 9 - DNA, 21 bp, Artificial Sequence
  source 1..21: mol_type = unassigned DNA
cacagaggcagagctgattgc

SEQ ID NO: 10 - DNA, 23 bp, Artificial Sequence
  source 1..23: mol_type = unassigned DNA
ccaattgaggagagtgacaggtt

SEQ ID NO: 11 - DNA, 21 bp, Artificial Sequence
  source 1..21: mol_type = unassigned DNA
agctgggcagaatacgtgctt

SEQ ID NO: 12 - DNA, 22 bp, Artificial Sequence
  source 1..22: mol_type = unassigned DNA
agaacaggcagaggagaatcca

SEQ ID NO: 13 - DNA, 20 bp, Artificial Sequence
  source 1..20: mol_type = unassigned DNA
tgtcctttcgaagccgttct

SEQ ID NO: 14 - DNA, 19 bp, Artificial Sequence
  source 1..19: mol_type = unassigned DNA
tgcagccagagtgcaagtg

SEQ ID NO: 15 - DNA, 20 bp, Artificial Sequence
  source 1..20: mol_type = unassigned DNA
agcgcaggctcaagaaagtg

SEQ ID NO: 16 - DNA, 19 bp, Artificial Sequence
  source 1..19: mol_type = unassigned DNA
ccgcctctgtagcggagat

SEQ ID NO: 17 - DNA, 23 bp, Artificial Sequence
  source 1..23: mol_type = unassigned DNA
gatcaccacgaacccatatgatt

SEQ ID NO: 18 - DNA, 23 bp, Artificial Sequence
  source 1..23: mol_type = unassigned DNA
ttcatgttcccataatgcatcac

SEQ ID NO: 19 - DNA, 20 bp, Artificial Sequence
  source 1..20: mol_type = unassigned DNA
ttcccatgttaccgctggat

SEQ ID NO: 20 - DNA, 22 bp, Artificial Sequence
  source 1..22: mol_type = unassigned DNA
gctgcttgaggatgtgaatttg

SEQ ID NO: 21 - DNA, 21 bp, Artificial Sequence
  source 1..21: mol_type = unassigned DNA
ctgcaccaccaactgcttagc

SEQ ID NO: 22 - DNA, 20 bp, Artificial Sequence
  source 1..20: mol_type = unassigned DNA
tcttctgggtggcagtgatg

SEQ ID NO: 23 - DNA, 25 bp, Artificial Sequence
  source 1..25: mol_type = unassigned DNA
ggaactactccagaccctctacaca

SEQ ID NO: 24 - DNA, 21 bp, Artificial Sequence
  source 1..21: mol_type = unassigned DNA
ctccatccgatacacccacat

SEQ ID NO: 25 - DNA, 23 bp, Artificial Sequence
  source 1..23: mol_type = unassigned DNA
ttgactttgggacagatgaggaa

SEQ ID NO: 26 - DNA, 22 bp, Artificial Sequence
  source 1..22: mol_type = unassigned DNA
ccagctccttactggtgtcctt